European Patent Application EP 4 624 584 A1, published October 1, 2025. Title: Helper Gene Control. Applicant: 株式会社シンプロジェン. The sequence listing filed with the application follows.

SEQUENCE LISTING (131 sequences)

SEQ ID NO: 1 - DNA, 20 bp, synthetic construct
  misc_feature 1..20: note = primer
  source 1..20: mol_type = other DNA
cctacggcgctctggatatg

SEQ ID NO: 2 - DNA, 22 bp, synthetic construct
  misc_feature 1..22: note = primer
  source 1..22: mol_type = other DNA
tacccaccgtactcgtcaattc

SEQ ID NO: 3 - DNA, 21 bp, synthetic construct
  misc_feature 1..21: note = primer
  source 1..21: mol_type = other DNA
atggaggcttgggagtgtttg

SEQ ID NO: 4 - DNA, 22 bp, synthetic construct
  misc_feature 1..22: note = primer
  source 1..22: mol_type = other DNA
actaactttgcctgggatgagc

SEQ ID NO: 5 - DNA, 22 bp, synthetic construct
  misc_feature 1..22: note = primer
  source 1..22: mol_type = other DNA
tctgccacggaggtgttattac

SEQ ID NO: 6 - DNA, 22 bp, synthetic construct
  misc_feature 1..22: note = primer
  source 1..22: mol_type = other DNA
cagccagtacctcttcgatcag

SEQ ID NO: 7 - DNA, 20 bp, synthetic construct
  misc_feature 1..20: note = primer
  source 1..20: mol_type = other DNA
catcaatgggcgtggatagc

SEQ ID NO: 8 - DNA, 24 bp, synthetic construct
  misc_feature 1..24: note = primer
  source 1..24: mol_type = other DNA
ggagttgttacgacattttggaaa

SEQ ID NO: 9 - DNA, 20 bp, synthetic construct
  misc_feature 1..20: note = primer
  source 1..20: mol_type = other DNA
cacccactcctccacctttg

SEQ ID NO: 10 - DNA, 23 bp, synthetic construct
  misc_feature 1..23: note = primer
  source 1..23: mol_type = other DNA
gccaaattcgttgtcataccagg

SEQ ID NO: 11 - DNA, 22 bp, synthetic construct
  misc_feature 1..22: note = primer
  source 1..22: mol_type = other DNA
gaaggtgctgaggtacgatgag

SEQ ID NO: 12 - DNA, 21 bp, synthetic construct
  misc_feature 1..21: note = primer
  source 1..21: mol_type = other DNA
ggtcacatccagcatcacagg

SEQ ID NO: 13 - DNA, 22 bp, synthetic construct
  misc_feature 1..22: note = primer
  source 1..22: mol_type = other DNA
tgacagctttgtgaactgggtg

SEQ ID NO: 14 - DNA, 22 bp, synthetic construct
  misc_feature 1..22: note = primer
  source 1..22: mol_type = other DNA
cgtgcatgtggaagtagctctc

SEQ ID NO: 15 - DNA, 52 bp, synthetic construct
  misc_feature 1..52: note = primer
  source 1..52: mol_type = other DNA
ttagtaagcttccctcctgacgcggtaggaggaggggagggtgccctgcatg

SEQ ID NO: 16 - DNA, 56 bp, synthetic construct
  misc_feature 1..56: note = primer
  source 1..56: mol_type = other DNA
ccttttgctcacatgtcaattggtagatgtacctggacatccaggtgatgccggcg

SEQ ID NO: 17 - DNA, 60 bp, synthetic construct
  misc_feature 1..60: note = primer
  source 1..60: mol_type = other DNA
tgtacaggcgcgccgaattcgttttagggcggagtaacttgtatgtgttgggaattgtag

SEQ ID NO: 18 - DNA, 51 bp, synthetic construct
  misc_feature 1..51: note = primer
  source 1..51: mol_type = other DNA
agggaagcttactaaacggtacacaggaaacaggagacacaactccaagtg

SEQ ID NO: 19 - DNA, 76 bp, synthetic construct
  misc_feature 1..76: note = primer
  source 1..76: mol_type = other DNA
gaaaagtgccacctgacgtcgcggccgcgcgatcgcggtacccaactccatgctcaacagtccccaggtacagccc

SEQ ID NO: 20 - DNA, 60 bp, synthetic construct
  misc_feature 1..60: note = primer
  source 1..60: mol_type = other DNA
gaattcggcgcgcctgtacagcccgggcgaccgcaccctgtgacgaaagccgcccgcaag

SEQ ID NO: 21 - DNA, 108 bp, synthetic construct
  misc_feature 1..108: note = primer
  source 1..108: mol_type = other DNA
gaaaagtgccacctgacgtcgcggccgcggaggggtggagtcgtgacgtgaattacgtcatagggttagggaggtcctgtattagaggtcacgtgagtgttttgcgac

SEQ ID NO: 22 - DNA, 99 bp, synthetic construct
  misc_feature 1..99: note = primer
  source 1..99: mol_type = other DNA
gttcaaacctcccgcttcaaaatggagaccctgcgtgctcactcgggcttaaatacccagcgtgaccacatggtgtcgcaaaatgtcgcaaaacactca

SEQ ID NO: 23 - DNA, 41 bp, synthetic construct
  misc_feature 1..41: note = primer
  source 1..41: mol_type = other DNA
gcgggaggtttgaacgcgcagccgccatgccggggttttac

SEQ ID NO: 24 - DNA, 38 bp, synthetic construct
  misc_feature 1..38: note = primer
  source 1..38: mol_type = other DNA
gatcgcagcgctatttaaatcatttattgttcaaagat

SEQ ID NO: 25 - DNA, 32 bp, synthetic construct
  misc_feature 1..32: note = primer
  source 1..32: mol_type = other DNA
aatagcgctgcgatcgcggcctccaaaaaagc

SEQ ID NO: 26 - DNA, 37 bp, synthetic construct
  misc_feature 1..37: note = primer
  source 1..37: mol_type = other DNA
ccttttgctcacatgtcaattgatcccgcccctaact

SEQ ID NO: 27 - DNA, 23 bp, synthetic construct
  misc_feature 1..23: note = primer
  source 1..23: mol_type = other DNA
aacaataaatgatttaaatcagg

SEQ ID NO: 28 - DNA, 38 bp, synthetic construct
  misc_feature 1..38: note = primer
  source 1..38: mol_type = other DNA
ggccgcgatcgcagcgctgtagccatggaaactagata

SEQ ID NO: 29 - DNA, 52 bp, synthetic construct
  misc_feature 1..52: note = primer
  source 1..52: mol_type = other DNA
gtgccacctgacgtcggccggccgcggccgcggtaccgagctcgactttcac

SEQ ID NO: 30 - DNA, 42 bp, synthetic construct
  misc_feature 1..42: note = primer
  source 1..42: mol_type = other DNA
tggtcctcctggatccgctagccaattcggggccgcggaggc

SEQ ID NO: 31 - DNA, 29 bp, synthetic construct
  misc_feature 1..29: note = primer
  source 1..29: mol_type = other DNA
ggggctagcatgccggggttttacgagat

SEQ ID NO: 32 - DNA, 29 bp, synthetic construct
  misc_feature 1..29: note = primer
  source 1..29: mol_type = other DNA
cccggatccactgcttctccgaggtaatc

SEQ ID NO: 33 - DNA, 22 bp, synthetic construct
  misc_feature 1..22: note = primer
  source 1..22: mol_type = other DNA
atcaagtgtatcatatgccaag

SEQ ID NO: 34 - DNA, 30 bp, synthetic construct
  misc_feature 1..30: note = primer
  source 1..30: mol_type = other DNA
tctagacatggtggcatctgacggttcact

SEQ ID NO: 35 - DNA, 18 bp, synthetic construct
  misc_feature 1..18: note = primer
  source 1..18: mol_type = other DNA
gatgccaccatgtctaga

SEQ ID NO: 36 - DNA, 30 bp, synthetic construct
  misc_feature 1..30: note = primer
  source 1..30: mol_type = other DNA
gcgggaattcccgatctacccaccgtactc

SEQ ID NO: 37 - DNA, 18 bp, synthetic construct
  misc_feature 1..18: note = primer
  source 1..18: mol_type = other DNA
agatcgggaattcccgcg

SEQ ID NO: 38 - DNA, 26 bp, synthetic construct
  misc_feature 1..26: note = primer
  source 1..26: mol_type = other DNA
ctttttcatggtggccacgtgaggtc

SEQ ID NO: 39 - DNA, 22 bp, synthetic construct
  misc_feature 1..22: note = primer
  source 1..22: mol_type = other DNA
gccaccatgaaaaagcctgaac

SEQ ID NO: 40 - DNA, 35 bp, synthetic construct
  misc_feature 1..35: note = primer
  source 1..35: mol_type = other DNA
tcattggtcttaaaggtaccctattcctttgccct

SEQ ID NO: 41 - DNA, 31 bp, synthetic construct
  misc_feature 1..31: note = primer
  source 1..31: mol_type = other DNA
cgacggtatcgctagcttttaaaagaaaagg

SEQ ID NO: 42 - DNA, 34 bp, synthetic construct
  misc_feature 1..34: note = primer
  source 1..34: mol_type = other DNA
tacaaagttgggatccatccgataatcactagta

SEQ ID NO: 43 - DNA, 25 bp, synthetic construct
  misc_feature 1..25: note = primer
  source 1..25: mol_type = other DNA
tggatcccaactttgtatagaaaag

SEQ ID NO: 44 - DNA, 38 bp, synthetic construct
  misc_feature 1..38: note = primer
  source 1..38: mol_type = other DNA
ctacccggtagaattcctcgagagcctgcttttttgta

SEQ ID NO: 45 - DNA, 55 bp, synthetic construct
  misc_feature 1..55: note = primer
  source 1..55: mol_type = other DNA
attatcggatggatcctagtgtggcggaagtgtgatgttgcaagtgtggcggaac

SEQ ID NO: 46 - DNA, 55 bp, synthetic construct
  misc_feature 1..55: note = primer
  source 1..55: mol_type = other DNA
ctacccggtagaattctcaatctgtatcttcatcgctagagccaaactcagcgcg

SEQ ID NO: 47 - DNA, 56 bp, synthetic construct
  misc_feature 1..56: note = primer
  source 1..56: mol_type = other DNA
aaagcaggctctcgagatggaggcttgggagtgtttggaagatttttctgctgtgc

SEQ ID NO: 48 - DNA, 56 bp, synthetic construct
  misc_feature 1..56: note = primer
  source 1..56: mol_type = other DNA
ctacccggtagaattctcaatctgtatcttcatcgctagagccaaactcagcgcgg

SEQ ID NO: 49 - DNA, 56 bp, synthetic construct
  misc_feature 1..56: note = primer
  source 1..56: mol_type = other DNA
cctacccggtagaattctcattcccgagggtccaggccggctctcgggttccatgg

SEQ ID NO: 50 - DNA, 39 bp, synthetic construct
  misc_feature 1..39: note = primer
  source 1..39: mol_type = other DNA
gcctttcgacctcacgtggccaccatggccaagcctttg

SEQ ID NO: 51 - DNA, 38 bp, synthetic construct
  misc_feature 1..38: note = primer
  source 1..38: mol_type = other DNA
ggctaagatctacagctgttagccctcccacacataac

SEQ ID NO: 52 - DNA, 56 bp, synthetic construct
  misc_feature 1..56: note = primer
  source 1..56: mol_type = other DNA
aaagcaggctctcgagatgagacatattatctgccacggaggtgttattaccgaag

SEQ ID NO: 53 - DNA, 56 bp, synthetic construct
  misc_feature 1..56: note = primer
  source 1..56: mol_type = other DNA
ctacccggtagaattcttatggcctggggcgtttacagctcaagtccaaaggttgc

SEQ ID NO: 54 - DNA, 56 bp, synthetic construct
  misc_feature 1..56: note = primer
  source 1..56: mol_type = other DNA
aaagcaggctctcgagatggagcgaagaaacccatctgagcggggggtacctgctg

SEQ ID NO: 55 - DNA, 53 bp, synthetic construct
  misc_feature 1..53: note = primer
  source 1..53: mol_type = other DNA
ctacccggtagaattcgtcgactcaatctgtatcttcatcgctagagccaaac

SEQ ID NO: 56 - DNA, 51 bp, synthetic construct
  misc_feature 1..51: note = primer
  source 1..51: mol_type = other DNA
tacagattgagtcgacatgagacatattatctgccacggaggtgttattac

SEQ ID NO: 57 - DNA, 40 bp, synthetic construct
  misc_feature 1..40: note = primer
  source 1..40: mol_type = other DNA
gcgatgaagatacagattgagcccctctccctcccccccc

SEQ ID NO: 58 - DNA, 40 bp, synthetic construct
  misc_feature 1..40: note = primer
  source 1..40: mol_type = other DNA
tggcagataatatgtctcatggttgtggccatattatcat

SEQ ID NO: 59 - DNA, 31 bp, synthetic construct
  misc_feature 1..31: note = primer
  source 1..31: mol_type = other DNA
tcaccatcttgtcgacacagtcgttgaaggg

SEQ ID NO: 60 - DNA, 44 bp, synthetic construct
  misc_feature 1..44: note = primer
  source 1..44: mol_type = other DNA
agcgcagcgagtcggccggccgcggccgcggaggggtggagtcg

SEQ ID NO: 61 - DNA, 40 bp, synthetic construct
  misc_feature 1..40: note = primer
  source 1..40: mol_type = other DNA
gcgatgaagatacagattgaggtactgaaatgtgtgggcg

SEQ ID NO: 62 - DNA, 62 bp, synthetic construct
  misc_feature 1..62: note = primer
  source 1..62: mol_type = other DNA
ctcccctacccggtagaattcagacagcaagacacttgcttgatccaaatccaaacagagtc

SEQ ID NO: 63 - DNA, 42 bp, synthetic construct
  misc_feature 1..42: note = primer
  source 1..42: mol_type = other DNA
cttgctgtctgaattctaggttctaccgggtaggggaggcgc

SEQ ID NO: 64 - DNA, 46 bp, synthetic construct
  misc_feature 1..46: note = primer
  source 1..46: mol_type = other DNA
gcggccgcagatctacgcgtgtcgacaaggacagggaagggagcag

SEQ ID NO: 65 - DNA, 35 bp, synthetic construct
  misc_feature 1..35: note = primer
  source 1..35: mol_type = other DNA
tagatctgcggccgcgagcaaaaggccagcaaaag

SEQ ID NO: 66 - DNA, 49 bp, synthetic construct
  misc_feature 1..49: note = primer
  source 1..49: mol_type = other DNA
cgccacactaggatccaagcttgcggccgcaggtggcacttttcgggga

SEQ ID NO: 67 - DNA, 55 bp, synthetic construct
  misc_feature 1..55: note = primer
  source 1..55: mol_type = other DNA
cgaaaagtgccacctgcggccgcaagctttctaggcgttacataacttacggtaa

SEQ ID NO: 68 - DNA, 42 bp, synthetic construct
  misc_feature 1..42: note = primer
  source 1..42: mol_type = other DNA
gaattccctgcagggctcttcagctctgcttatatagacctc

SEQ ID NO: 69 - DNA, 32 bp, synthetic construct
  misc_feature 1..32: note = primer
  source 1..32: mol_type = other DNA
ccctgcagggaattctaagatacattgatgag

SEQ ID NO: 70 - DNA, 31 bp, synthetic construct
  misc_feature 1..31: note = primer
  source 1..31: mol_type = other DNA
ggaggatccaacttgtttattgcagcttata

SEQ ID NO: 71 - DNA, 33 bp, synthetic construct
  misc_feature 1..33: note = primer
  source 1..33: mol_type = other DNA
caagttggatcctccccagcatgcctgctattc

SEQ ID NO: 72 - DNA, 33 bp, synthetic construct
  misc_feature 1..33: note = primer
  source 1..33: mol_type = other DNA
ttggctagctgtacactgtgccttctagttgcc

SEQ ID NO: 73 - DNA, 33 bp, synthetic construct; identical to SEQ ID NO: 71
  misc_feature 1..33: note = primer
  source 1..33: mol_type = other DNA

SEQ ID NO: 74 - DNA, 60 bp, synthetic construct
  misc_feature 1..60: note = primer
  source 1..60: mol_type = other DNA
gctggccttttgctcgcggccgcagatctacgcgtcctaggctcgacattgattattgac

SEQ ID NO: 75 - DNA, 31 bp, synthetic construct
  misc_feature 1..31: note = primer
  source 1..31: mol_type = other DNA
gccctgcagggaattcatgagacatattatc

SEQ ID NO: 76 - DNA, 35 bp, synthetic construct
  misc_feature 1..35: note = primer
  source 1..35: mol_type = other DNA
atgtatcttagaattttatggcctggggcgtttac

SEQ ID NO: 77 - DNA, 37 bp, synthetic construct
  misc_feature 1..37: note = primer
  source 1..37: mol_type = other DNA
caaagaattggctagcatggaggcttgggagtgtttg

SEQ ID NO: 78 - DNA, 35 bp, synthetic construct
  misc_feature 1..35: note = primer
  source 1..35: mol_type = other DNA
acagtgtacagctagtcaatctgtatcttcatcgc

SEQ ID NO: 79 - DNA, 35 bp, synthetic construct
  misc_feature 1..35: note = primer
  source 1..35: mol_type = other DNA
cttgctgtctgaattctaggttctaccgggtaggg

SEQ ID NO: 80 - DNA, 22 bp, synthetic construct
  misc_feature 1..22: note = primer
  source 1..22: mol_type = other DNA
ccgcagatctacgcgtgtcgac

SEQ ID NO: 81 - DNA, 40 bp, synthetic construct
  misc_feature 1..40: note = primer
  source 1..40: mol_type = other DNA
tcccaagcctccatgctagccaattcggggccgcggaggc

SEQ ID NO: 82 - DNA, 42 bp, synthetic construct
  misc_feature 1..42: note = primer
  source 1..42: mol_type = other DNA
ccctacccggtagaacctaggcaactttgtatagaaaagttg

SEQ ID NO: 83 - DNA, 40 bp, synthetic construct
  misc_feature 1..40: note = primer
  source 1..40: mol_type = other DNA
ctgtccttgtcgacacgcgtgagcaaaaggccagcaaaag

SEQ ID NO: 84 - DNA, 42 bp, synthetic construct
  misc_feature 1..42: note = primer
  source 1..42: mol_type = other DNA
gataatatgtctcatgaattcagcctgcttttttgtacaaac

SEQ ID NO: 85 - DNA, 36 bp, synthetic construct
  misc_feature 1..36: note = primer
  source 1..36: mol_type = other DNA
cttgctgtctgaattctaggttctaccgggtagggg

SEQ ID NO: 86 - DNA, 27 bp, synthetic construct
  misc_feature 1..27: note = primer
  source 1..27: mol_type = other DNA
cgcggccgcagatctacgcgtgtcgac

SEQ ID NO: 87 - DNA, 37 bp, synthetic construct
  misc_feature 1..37: note = primer
  source 1..37: mol_type = other DNA
ccgcaagcttggatcccaactttgtatagaaaagttg

SEQ ID NO: 88 - DNA, 22 bp, synthetic construct
  misc_feature 1..22: note = primer
  source 1..22: mol_type = other DNA
tattgcattctctagacacagg

SEQ ID NO: 89 - DNA, 21 bp, synthetic construct
  misc_feature 1..21: note = primer
  source 1..21: mol_type = other DNA
attgcgtgtgtggttaacgcc

SEQ ID NO: 90 - DNA, 29 bp, synthetic construct
  misc_feature 1..29: note = primer
  source 1..29: mol_type = other DNA
ttctatacaaagttggaggtcagatgtaa

SEQ ID NO: 91 - DNA, 21 bp, synthetic construct
  misc_feature 1..21: note = primer
  source 1..21: mol_type = other DNA
caactttgtatagaaaagttg

SEQ ID NO: 92 - DNA, 23 bp, synthetic construct
  misc_feature 1..23: note = primer
  source 1..23: mol_type = other DNA
tccatttatcctttataaaactc

SEQ ID NO: 93 - DNA, 20 bp, synthetic construct
  source 1..20: mol_type = other DNA
  misc_feature 1..20: note = primer
tctgaagactacagcgtcgc

SEQ ID NO: 94 - DNA, 25 bp, synthetic construct
  source 1..25: mol_type = other DNA
  misc_feature 1..25: note = primer
ggtgtacaggatggaacatgaaggc

SEQ ID NO: 95 - DNA, 21 bp, synthetic construct
  source 1..21: mol_type = other DNA
  misc_feature 1..21: note = primer
acctgcgcttgtggtatgatg

SEQ ID NO: 96 - DNA, 22 bp, synthetic construct
  source 1..22: mol_type = other DNA
  misc_feature 1..22: note = primer
gtgcaaggcgctgtatccaaag

SEQ ID NO: 97 - DNA, 20 bp, synthetic construct
  source 1..20: mol_type = other DNA
  misc_feature 1..20: note = primer
atctccttcaatgcggcctc

SEQ ID NO: 98 - DNA, 20 bp, synthetic construct
  source 1..20: mol_type = other DNA
  misc_feature 1..20: note = primer
agacggaagccgcatattgg

SEQ ID NO: 99 - DNA, 20 bp, synthetic construct
  source 1..20: mol_type = other DNA
  misc_feature 1..20: note = primer
atgagacatattatctgcca

SEQ ID NO: 100 - DNA, 20 bp, synthetic construct
  source 1..20: mol_type = other DNA
  misc_feature 1..20: note = primer
gccaaactcagcgcgggtgc

SEQ ID NO: 101 - DNA, 62 bp, synthetic construct
  source 1..62: mol_type = other DNA
  misc_feature 1..62: note = primer
ttcaggttggaccggtgccaccatgccgaagaaaaagcgcaaggtcgaagcgtccgacaaga

SEQ ID NO: 102 - DNA, 60 bp, synthetic construct
  source 1..60: mol_type = other DNA
  misc_feature 1..60: note = primer
cccacagagttggtgccgatggccaggccgatgctgtacttcttgtcggacgcttcgacc

SEQ ID NO: 103 - DNA, 23 bp, synthetic construct
  source 1..23: mol_type = other DNA
  misc_feature 1..23: note = primer
gccatcggcaccaactctgtggg

SEQ ID NO: 104 - DNA, 23 bp, synthetic construct
  source 1..23: mol_type = other DNA
  misc_feature 1..23: note = primer
tcgttgctgaagatctcttgcag

SEQ ID NO: 105 - DNA, 24 bp, synthetic construct
  source 1..24: mol_type = other DNA
  misc_feature 1..24: note = primer
aggaacatccccttccctcggatg

SEQ ID NO: 106 - DNA, 23 bp, synthetic construct
  source 1..23: mol_type = other DNA
  misc_feature 1..23: note = primer
aaaggtgaggcggctccggagaa

SEQ ID NO: 107 - DNA, 41 bp, synthetic construct
  source 1..41: mol_type = other DNA
  misc_feature 1..41: note = primer
cggcgcgccgcggccgcaggaacatccccttccctcggatg

SEQ ID NO: 108 - DNA, 45 bp, synthetic construct
  source 1..45: mol_type = other DNA
  misc_feature 1..45: note = primer
cgccacactaggatcaagtcatcaacttgttatcctggtttacag

SEQ ID NO: 109 - DNA, 31 bp, synthetic construct
  source 1..31: mol_type = other DNA
  misc_feature 1..31: note = primer
gacttgatcctagtgtggcggaagtgtgatg

SEQ ID NO: 110 - DNA, 51 bp, synthetic construct
  source 1..51: mol_type = other DNA
  misc_feature 1..51: note = primer
tcacgccgccgtgacagatgatgtgccgcattttcagtcccggtgtcggag

SEQ ID NO: 111 - DNA, 59 bp, synthetic construct
  source 1..59: mol_type = other DNA
  misc_feature 1..59: note = primer
tcatctgtcacggcggcgtgatcacagaggaaatggccgccagtcttttggaccagctg

SEQ ID NO: 112 - DNA, 44 bp, synthetic construct
  source 1..44: mol_type = other DNA
  misc_feature 1..44: note = primer
gcaaacaaaggcgttaaccacacacgcaatcacaggtttacacc

SEQ ID NO: 113 - DNA, 88 bp, synthetic construct
  source 1..88: mol_type = other DNA
  misc_feature 1..88: note = primer
attgcgtgtgtggttaacgcctttgtttgctgaatgagttgatgtaagtttaataaacaactttgtatagaaaagttgggtaccgagc

SEQ ID NO: 114 - DNA, 30 bp, synthetic construct
  source 1..30: mol_type = other DNA
  misc_feature 1..30: note = primer
tcccaagcctccatgctagccaattcgggg

SEQ ID NO: 115 - DNA, 30 bp, synthetic construct
  source 1..30: mol_type = other DNA
  misc_feature 1..30: note = primer
ccttgggtatcctgtctgagggtaactcca

SEQ ID NO: 116 - DNA, 53 bp, synthetic construct
  source 1..53: mol_type = other DNA
  misc_feature 1..53: note = primer
gtcggagctgccaaactcggctctggtacaggccagcaccaagtgatcgggcc

SEQ ID NO: 117 - DNA, 53 bp, synthetic construct
  source 1..53: mol_type = other DNA
  misc_feature 1..53: note = primer
gagtttggcagctccgacgaggacaccgattgaggtactgaaatgtgtgggcg

SEQ ID NO: 118 - DNA, 35 bp, synthetic construct
  source 1..35: mol_type = other DNA
  misc_feature 1..35: note = primer
gccggttggcgcctaccggtggatgtggaatgtgt

SEQ ID NO: 119 - DNA, 20 bp, synthetic construct
  source 1..20: mol_type = other DNA
  misc_feature 1..20: note = primer
gataaatatgtggccggggg

SEQ ID NO: 120 - DNA, 25 bp, synthetic construct
  source 1..25: mol_type = other DNA
  misc_feature 1..25: note = primer
tgaccactgaagcacagcatcacag

SEQ ID NO: 121 - DNA, 41 bp, synthetic construct
  source 1..41: mol_type = other DNA
  misc_feature 1..41: note = primer
ccctgtccttgtcgaccaaagatgtcagaacaagactcccc

SEQ ID NO: 122 - DNA, 41 bp, synthetic construct
  source 1..41: mol_type = other DNA
  misc_feature 1..41: note = primer
ccttttgctcacgcgttgaccactgaagcacagcatcacag

SEQ ID NO: 123 - DNA, 23 bp, synthetic construct
  source 1..23: mol_type = other DNA
  misc_feature 1..23: note = primer
tcagcagcagccgcgggcccttg

SEQ ID NO: 124 - DNA, 20 bp, synthetic construct
  source 1..20: mol_type = other DNA
  misc_feature 1..20: note = primer
gcccgggcgaccgcaccctg

SEQ ID NO: 125 - DNA, 50 bp, synthetic construct
  source 1..50: mol_type = other DNA
  misc_feature 1..50: note = primer
agggtgcggtcgcccgggcgttttagggcggagtaacttgtatgtgttgg

SEQ ID NO: 126 - DNA, 30 bp, synthetic construct
  source 1..30: mol_type = other DNA
  misc_feature 1..30: note = primer
ggttaactccccagcatgcctgctattctc

SEQ ID NO: 127 - DNA, 45 bp, synthetic construct
  misc_feature 1..45: note = primer
  source 1..45: mol_type = other DNA
gcaggcatgctggggagttaacccctcctgacgcggtaggaggag

SEQ ID NO: 128 - DNA, 36 bp, synthetic construct
  source 1..36: mol_type = other DNA
  misc_feature 1..36: note = primer
tcgttgacgctctagaccgtgcaaaaggagagcctg

SEQ ID NO: 129 - DNA, 49 bp, synthetic construct
  source 1..49: mol_type = other DNA
  misc_feature 1..49: note = primer
agggtgcggtcgcccgggccaactttgtatagaaaagttgggtaccgag

SEQ ID NO: 130 - DNA, 40 bp, synthetic construct
  source 1..40: mol_type = other DNA
  misc_feature 1..40: note = primer
ggaacgccggacgtagtcatcaattcggggccgcggaggc

SEQ ID NO: 131 - DNA, 26 bp, synthetic construct
  source 1..26: mol_type = other DNA
  misc_feature 1..26: note = primer
atgactacgtccggcgttccatttgg